European Patent Application EP 4 578 464 A1, published July 2, 2025. Title: 抗体偶联药物的药物组合物. Applicant: 启德医药科技（苏州）有限公司. Application CN. The sequence listing filed with the application follows.

SEQUENCE LISTING (4 sequences)

SEQ ID NO: 1 - protein, 222 aa, synthetic construct
DIQMTQSPSSLSASVGDRVTITCRASQDVNTAVAWYQQKPGKAPKLLIYSASFLYSGVPSRFSGSRSGTDFTLTISSLQPEDFATYYCQQHYTTPPTFGQGTKVEIKRTVAAPSVFIFPPSDEQLKSGTASVVCLLNNFYPREAKVQWKVDNALQSGNSQESVTEQDSKDSTYSLSSTLTLSKADYEKHKVYACEVTHQGLSSPVTKSFNRGECGALPETGG

SEQ ID NO: 2 - protein, 450 aa, synthetic construct
EVQLVESGGGLVQPGGSLRLSCAASGFNIKDTYIHWVRQAPGKGLEWVARIYPTNGYTRYADSVKGRFTISADTSKNTAYLQMNSLRAEDTAVYYCSRWGGDGFYAMDYWGQGTLVTVSSASTKGPSVFPLAPSSKSTSGGTAALGCLVKDYFPEPVTVSWNSGALTSGVHTFPAVLQSSGLYSLSSVVTVPSSSLGTQTYICNVNHKPSNTKVDKKVEPKSCDKTHTCPPCPAPELLGGPSVFLFPPKPKDTLMISRTPEVTCVVVDVSHEDPEVKFNWYVDGVEVHNAKTKPREEQYNSTYRVVSVLTVLHQDWLNGKEYKCKVSNKALPAPIEKTISKAKGQPREPQVYTLPPSREEMTKNQVSLTCLVKGFYPSDIAVEWESNGQPENNYKTTPPVLDSDGSFFLYSKLTVDKSRWQQGNVFSCSVMHEALHNHYTQKSLSLSPGK

SEQ ID NO: 3 - protein, 222 aa, synthetic construct; identical to SEQ ID NO: 1

SEQ ID NO: 4 - protein, 458 aa, synthetic construct
EVQLVESGGGLVQPGGSLRLSCAASGFNIKDTYIHWVRQAPGKGLEWVARIYPTNGYTRYADSVKGRFTISADTSKNTAYLQMNSLRAEDTAVYYCSRWGGDGFYAMDYWGQGTLVTVSSASTKGPSVFPLAPSSKSTSGGTAALGCLVKDYFPEPVTVSWNSGALTSGVHTFPAVLQSSGLYSLSSVVTVPSSSLGTQTYICNVNHKPSNTKVDKKVEPKSCDKTHTCPPCPAPELLGGPSVFLFPPKPKDTLMISRTPEVTCVVVDVSHEDPEVKFNWYVDGVEVHNAKTKPREEQYNSTYRVVSVLTVLHQDWLNGKEYKCKVSNKALPAPIEKTISKAKGQPREPQVYTLPPSREEMTKNQVSLTCLVKGFYPSDIAVEWESNGQPENNYKTTPPVLDSDGSFFLYSKLTVDKSRWQQGNVFSCSVMHEALHNHYTQKSLSLSPGKGALPETGG